European Patent Application EP 4 692 347 A1, published February 11, 2026. Title: DSRNA MOLECULE FOR REGULATING EXPRESSION OF CIDEB MRNA. Applicant: Rona Bioscience, Limited. The sequence listing filed with the application follows.

SEQUENCE LISTING (388 sequences)

SEQ ID NO: 1 - RNA, 19 nt, synthetic construct
  source 1..19: mol_type = other RNA
caccatggagtacctctca

SEQ ID NO: 2 - RNA, 19 nt, synthetic construct
  source 1..19: mol_type = other RNA
gctctgaaccccagtgact

SEQ ID NO: 3 - RNA, 19 nt, synthetic construct
  source 1..19: mol_type = other RNA
tactcaggtcagtatctaa

SEQ ID NO: 4 - RNA, 19 nt, synthetic construct
  source 1..19: mol_type = other RNA
aggtcagtatctaatataa

SEQ ID NO: 5 - RNA, 19 nt, synthetic construct
  source 1..19: mol_type = other RNA
gccaggagctgctagccaa

SEQ ID NO: 6 - RNA, 19 nt, synthetic construct
  source 1..19: mol_type = other RNA
cctttgacgtgtacaagca

SEQ ID NO: 7 - RNA, 19 nt, synthetic construct
  source 1..19: mol_type = other RNA
ctctatgagttgtgacttt

SEQ ID NO: 8 - RNA, 19 nt, synthetic construct
  source 1..19: mol_type = other RNA
gccatatgttgctgggaat

SEQ ID NO: 9 - RNA, 19 nt, synthetic construct
  source 1..19: mol_type = other RNA
ccgcctccattcctactaa

SEQ ID NO: 10 - RNA, 19 nt, synthetic construct
  source 1..19: mol_type = other RNA
gcaaagactatgacagcat

SEQ ID NO: 11 - RNA, 19 nt, synthetic construct
  source 1..19: mol_type = other RNA
agactatgacagcatcaaa

SEQ ID NO: 12 - RNA, 19 nt, synthetic construct
  source 1..19: mol_type = other RNA
gactatgacagcatcaaat

SEQ ID NO: 13 - RNA, 19 nt, synthetic construct
  source 1..19: mol_type = other RNA
actatgacagcatcaaatt

SEQ ID NO: 14 - RNA, 19 nt, synthetic construct
  source 1..19: mol_type = other RNA
ctatgacagcatcaaattt

SEQ ID NO: 15 - RNA, 19 nt, synthetic construct
  source 1..19: mol_type = other RNA
atgacagcatcaaatttca

SEQ ID NO: 16 - RNA, 19 nt, synthetic construct
  source 1..19: mol_type = other RNA
tgacagcatcaaatttcaa

SEQ ID NO: 17 - RNA, 19 nt, synthetic construct
  source 1..19: mol_type = other RNA
cagacagtacaggctagat

SEQ ID NO: 18 - RNA, 19 nt, synthetic construct
  source 1..19: mol_type = other RNA
agacagtacaggctagata

SEQ ID NO: 19 - RNA, 19 nt, synthetic construct
  source 1..19: mol_type = other RNA
gacagtacaggctagataa

SEQ ID NO: 20 - RNA, 19 nt, synthetic construct
  source 1..19: mol_type = other RNA
aaacatttccaataaaaat

SEQ ID NO: 21 - RNA, 19 nt, synthetic construct
  source 1..19: mol_type = other RNA
acatttccaataaaaatat

SEQ ID NO: 22 - RNA, 19 nt, synthetic construct
  source 1..19: mol_type = other RNA
ctctgaaccccagtgactt

SEQ ID NO: 23 - RNA, 19 nt, synthetic construct
  source 1..19: mol_type = other RNA
gacctttccgtgtctgtga

SEQ ID NO: 24 - RNA, 19 nt, synthetic construct
  source 1..19: mol_type = other RNA
cctcacatcccaagtctat

SEQ ID NO: 25 - RNA, 19 nt, synthetic construct
  source 1..19: mol_type = other RNA
ccctaaactccccagcata

SEQ ID NO: 26 - RNA, 19 nt, synthetic construct
  source 1..19: mol_type = other RNA
atttccaataaaaatatca

SEQ ID NO: 27 - RNA, 19 nt, synthetic construct
  source 1..19: mol_type = other RNA
cccttacctgaagaatgct

SEQ ID NO: 28 - RNA, 19 nt, synthetic construct
  source 1..19: mol_type = other RNA
tcacatcccaagtctataa

SEQ ID NO: 29 - RNA, 19 nt, synthetic construct
  source 1..19: mol_type = other RNA
cttacctgaagaatgctgt

SEQ ID NO: 30 - RNA, 19 nt, synthetic construct
  source 1..19: mol_type = other RNA
tatgacagcatcaaattta

SEQ ID NO: 31 - RNA, 19 nt, synthetic construct
  source 1..19: mol_type = other RNA
gcctgactgctgctacata

SEQ ID NO: 32 - RNA, 19 nt, synthetic construct
  source 1..19: mol_type = other RNA
tacccttacctgaagaata

SEQ ID NO: 33 - RNA, 19 nt, synthetic construct
  source 1..19: mol_type = other RNA
ccttacctgaagaatgcta

SEQ ID NO: 34 - RNA, 19 nt, synthetic construct
  source 1..19: mol_type = other RNA
tagataacccacccaattt

SEQ ID NO: 35 - RNA, 19 nt, synthetic construct
  source 1..19: mol_type = other RNA
ctaaactccccagcatact

SEQ ID NO: 36 - RNA, 19 nt, synthetic construct
  source 1..19: mol_type = other RNA
cagcctgactgctgctaca

SEQ ID NO: 37 - RNA, 19 nt, synthetic construct
  source 1..19: mol_type = other RNA
acaaaaacatttccaataa

SEQ ID NO: 38 - RNA, 19 nt, synthetic construct
  source 1..19: mol_type = other RNA
actgctgaatggagtgcta

SEQ ID NO: 39 - RNA, 19 nt, synthetic construct
  source 1..19: mol_type = other RNA
acctttccgtgtctgtgat

SEQ ID NO: 40 - RNA, 19 nt, synthetic construct
  source 1..19: mol_type = other RNA
gacttactcaggtcagtat

SEQ ID NO: 41 - RNA, 19 nt, synthetic construct
  source 1..19: mol_type = other RNA
ctagataacccacccaatt

SEQ ID NO: 42 - RNA, 19 nt, synthetic construct
  source 1..19: mol_type = other RNA
accccagtgacttactcaa

SEQ ID NO: 43 - RNA, 19 nt, synthetic construct
  source 1..19: mol_type = other RNA
gtacctctcagctctgaaa

SEQ ID NO: 44 - RNA, 19 nt, synthetic construct
  source 1..19: mol_type = other RNA
acatcccaagtctatacca

SEQ ID NO: 45 - RNA, 19 nt, synthetic construct
  source 1..19: mol_type = other RNA
agtacaggctagataacca

SEQ ID NO: 46 - RNA, 19 nt, synthetic construct
  source 1..19: mol_type = other RNA
cttactcaggtcagtatct

SEQ ID NO: 47 - RNA, 19 nt, synthetic construct
  source 1..19: mol_type = other RNA
ctcaggtcagtatctaata

SEQ ID NO: 48 - RNA, 19 nt, synthetic construct
  source 1..19: mol_type = other RNA
ccccagaatcattccaaca

SEQ ID NO: 49 - RNA, 19 nt, synthetic construct
  source 1..19: mol_type = other RNA
cagcataacgcctcacata

SEQ ID NO: 50 - RNA, 19 nt, synthetic construct
  source 1..19: mol_type = other RNA
aacaaaaacatttccaata

SEQ ID NO: 51 - RNA, 19 nt, synthetic construct
  source 1..19: mol_type = other RNA
cctaaactccccagcataa

SEQ ID NO: 52 - RNA, 19 nt, synthetic construct
  source 1..19: mol_type = other RNA
aatataagctcggagttta

SEQ ID NO: 53 - RNA, 19 nt, synthetic construct
  source 1..19: mol_type = other RNA
tccctaaactccccagcat

SEQ ID NO: 54 - RNA, 19 nt, synthetic construct
  source 1..19: mol_type = other RNA
cccagtgacttactcaggt

SEQ ID NO: 55 - RNA, 19 nt, synthetic construct
  source 1..19: mol_type = other RNA
gtcagtatctaatataaga

SEQ ID NO: 56 - RNA, 19 nt, synthetic construct
  source 1..19: mol_type = other RNA
tacctctcagctctgaaca

SEQ ID NO: 57 - RNA, 19 nt, synthetic construct
  source 1..19: mol_type = other RNA
taaactccccagcatacta

SEQ ID NO: 58 - RNA, 19 nt, synthetic construct
  source 1..19: mol_type = other RNA
ggtgttgcagtctggtcaa

SEQ ID NO: 59 - RNA, 19 nt, synthetic construct
  source 1..19: mol_type = other RNA
gtgacttactcaggtcagt

SEQ ID NO: 60 - RNA, 19 nt, synthetic construct
  source 1..19: mol_type = other RNA
tgtcaaagccacattctaa

SEQ ID NO: 61 - RNA, 19 nt, synthetic construct
  source 1..19: mol_type = other RNA
ggacttggcccaaagaaaa

SEQ ID NO: 62 - RNA, 21 nt, synthetic construct
  source 1..21: mol_type = other RNA
tgagaggtactccatggtgga

SEQ ID NO: 63 - RNA, 21 nt, synthetic construct
  source 1..21: mol_type = other RNA
agtcactggggttcagagctg

SEQ ID NO: 64 - RNA, 21 nt, synthetic construct
  source 1..21: mol_type = other RNA
ttagatactgacctgagtaag

SEQ ID NO: 65 - RNA, 21 nt, synthetic construct
  source 1..21: mol_type = other RNA
ttatattagatactgacctga

SEQ ID NO: 66 - RNA, 21 nt, synthetic construct
  source 1..21: mol_type = other RNA
ttggctagcagctcctggctg

SEQ ID NO: 67 - RNA, 21 nt, synthetic construct
  source 1..21: mol_type = other RNA
tgcttgtacacgtcaaaggtg

SEQ ID NO: 68 - RNA, 21 nt, synthetic construct
  source 1..21: mol_type = other RNA
aaagtcacaactcatagagta

SEQ ID NO: 69 - RNA, 21 nt, synthetic construct
  source 1..21: mol_type = other RNA
attcccagcaacatatggctc

SEQ ID NO: 70 - RNA, 21 nt, synthetic construct
  source 1..21: mol_type = other RNA
ttagtaggaatggaggcggtc

SEQ ID NO: 71 - RNA, 21 nt, synthetic construct
  source 1..21: mol_type = other RNA
atgctgtcatagtctttgcag

SEQ ID NO: 72 - RNA, 21 nt, synthetic construct
  source 1..21: mol_type = other RNA
tttgatgctgtcatagtcttt

SEQ ID NO: 73 - RNA, 21 nt, synthetic construct
  source 1..21: mol_type = other RNA
atttgatgctgtcatagtctt

SEQ ID NO: 74 - RNA, 21 nt, synthetic construct
  source 1..21: mol_type = other RNA
aatttgatgctgtcatagtct

SEQ ID NO: 75 - RNA, 21 nt, synthetic construct
  source 1..21: mol_type = other RNA
aaatttgatgctgtcatagtc

SEQ ID NO: 76 - RNA, 21 nt, synthetic construct
  source 1..21: mol_type = other RNA
tgaaatttgatgctgtcatag

SEQ ID NO: 77 - RNA, 21 nt, synthetic construct
  source 1..21: mol_type = other RNA
ttgaaatttgatgctgtcata

SEQ ID NO: 78 - RNA, 21 nt, synthetic construct
  source 1..21: mol_type = other RNA
atctagcctgtactgtctgca

SEQ ID NO: 79 - RNA, 21 nt, synthetic construct
  source 1..21: mol_type = other RNA
tatctagcctgtactgtctgc

SEQ ID NO: 80 - RNA, 21 nt, synthetic construct
  source 1..21: mol_type = other RNA
ttatctagcctgtactgtctg

SEQ ID NO: 81 - RNA, 21 nt, synthetic construct
  source 1..21: mol_type = other RNA
atttttattggaaatgttttt

SEQ ID NO: 82 - RNA, 21 nt, synthetic construct
  source 1..21: mol_type = other RNA
atatttttattggaaatgttt

SEQ ID NO: 83 - RNA, 21 nt, synthetic construct
  source 1..21: mol_type = other RNA
aagtcactggggttcagagct

SEQ ID NO: 84 - RNA, 21 nt, synthetic construct
  source 1..21: mol_type = other RNA
tcacagacacggaaaggtcgc

SEQ ID NO: 85 - RNA, 21 nt, synthetic construct
  source 1..21: mol_type = other RNA
atagacttgggatgtgaggcg

SEQ ID NO: 86 - RNA, 21 nt, synthetic construct
  source 1..21: mol_type = other RNA
tatgctggggagtttagggac

SEQ ID NO: 87 - RNA, 21 nt, synthetic construct
  source 1..21: mol_type = other RNA
tgatatttttattggaaatgt

SEQ ID NO: 88 - RNA, 21 nt, synthetic construct
  source 1..21: mol_type = other RNA
agcattcttcaggtaagggta

SEQ ID NO: 89 - RNA, 21 nt, synthetic construct
  source 1..21: mol_type = other RNA
ttatagacttgggatgtgagg

SEQ ID NO: 90 - RNA, 21 nt, synthetic construct
  source 1..21: mol_type = other RNA
acagcattcttcaggtaaggg

SEQ ID NO: 91 - RNA, 21 nt, synthetic construct
  source 1..21: mol_type = other RNA
taaatttgatgctgtcatagt

SEQ ID NO: 92 - RNA, 21 nt, synthetic construct
  source 1..21: mol_type = other RNA
tatgtagcagcagtcaggctg

SEQ ID NO: 93 - RNA, 21 nt, synthetic construct
  source 1..21: mol_type = other RNA
tattcttcaggtaagggtata

SEQ ID NO: 94 - RNA, 21 nt, synthetic construct
  source 1..21: mol_type = other RNA
tagcattcttcaggtaagggt

SEQ ID NO: 95 - RNA, 21 nt, synthetic construct
  source 1..21: mol_type = other RNA
aaattgggtgggttatctagc

SEQ ID NO: 96 - RNA, 21 nt, synthetic construct
  source 1..21: mol_type = other RNA
agtatgctggggagtttaggg

SEQ ID NO: 97 - RNA, 21 nt, synthetic construct
  source 1..21: mol_type = other RNA
tgtagcagcagtcaggctggg

SEQ ID NO: 98 - RNA, 21 nt, synthetic construct
  source 1..21: mol_type = other RNA
ttattggaaatgtttttgtta

SEQ ID NO: 99 - RNA, 21 nt, synthetic construct
  source 1..21: mol_type = other RNA
tagcactccattcagcagtag

SEQ ID NO: 100 - RNA, 21 nt, synthetic construct
  source 1..21: mol_type = other RNA
atcacagacacggaaaggtcg

SEQ ID NO: 101 - RNA, 21 nt, synthetic construct
  source 1..21: mol_type = other RNA
atactgacctgagtaagtcac

SEQ ID NO: 102 - RNA, 21 nt, synthetic construct
  source 1..21: mol_type = other RNA
aattgggtgggttatctagcc

SEQ ID NO: 103 - RNA, 21 nt, synthetic construct
  source 1..21: mol_type = other RNA
ttgagtaagtcactggggttc

SEQ ID NO: 104 - RNA, 21 nt, synthetic construct
  source 1..21: mol_type = other RNA
tttcagagctgagaggtactc

SEQ ID NO: 105 - RNA, 21 nt, synthetic construct
  source 1..21: mol_type = other RNA
tggtatagacttgggatgtga

SEQ ID NO: 106 - RNA, 21 nt, synthetic construct
  source 1..21: mol_type = other RNA
tggttatctagcctgtactgt

SEQ ID NO: 107 - RNA, 21 nt, synthetic construct
  source 1..21: mol_type = other RNA
agatactgacctgagtaagtc

SEQ ID NO: 108 - RNA, 21 nt, synthetic construct
  source 1..21: mol_type = other RNA
tattagatactgacctgagta

SEQ ID NO: 109 - RNA, 21 nt, synthetic construct
  source 1..21: mol_type = other RNA
tgttggaatgattctgggggc

SEQ ID NO: 110 - RNA, 21 nt, synthetic construct
  source 1..21: mol_type = other RNA
tatgtgaggcgttatgctgaa

SEQ ID NO: 111 - RNA, 21 nt, synthetic construct
  source 1..21: mol_type = other RNA
tattggaaatgtttttgttag

SEQ ID NO: 112 - RNA, 21 nt, synthetic construct
  source 1..21: mol_type = other RNA
ttatgctggggagtttaggga

SEQ ID NO: 113 - RNA, 21 nt, synthetic construct
  source 1..21: mol_type = other RNA
taaactccgagcttatattag

SEQ ID NO: 114 - RNA, 21 nt, synthetic construct
  source 1..21: mol_type = other RNA
atgctggggagtttagggaca

SEQ ID NO: 115 - RNA, 21 nt, synthetic construct
  source 1..21: mol_type = other RNA
acctgagtaagtcactggggt

SEQ ID NO: 116 - RNA, 21 nt, synthetic construct
  source 1..21: mol_type = other RNA
tcttatattagatactgacct

SEQ ID NO: 117 - RNA, 21 nt, synthetic construct
  source 1..21: mol_type = other RNA
tgttcagagctgagaggtact

SEQ ID NO: 118 - RNA, 21 nt, synthetic construct
  source 1..21: mol_type = other RNA
tagtatgctggggagtttagg

SEQ ID NO: 119 - RNA, 21 nt, synthetic construct
  source 1..21: mol_type = other RNA
ttgaccagactgcaacaccat

SEQ ID NO: 120 - RNA, 21 nt, synthetic construct
  source 1..21: mol_type = other RNA
actgacctgagtaagtcactg

SEQ ID NO: 121 - RNA, 21 nt, synthetic construct
  source 1..21: mol_type = other RNA
ttagaatgtggctttgacatt

SEQ ID NO: 122 - RNA, 21 nt, synthetic construct
  source 1..21: mol_type = other RNA
ttttctttgggccaagtcctt

SEQ ID NO: 123 - RNA, 19 nt, synthetic construct
  source 1..19: mol_type = other RNA
caccatggagtacctctca

SEQ ID NO: 124 - RNA, 19 nt, synthetic construct
  source 1..19: mol_type = other RNA
gctctgaaccccagtgact

SEQ ID NO: 125 - RNA, 19 nt, synthetic construct
  source 1..19: mol_type = other RNA
tactcaggtcagtatctaa

SEQ ID NO: 126 - RNA, 19 nt, synthetic construct
  source 1..19: mol_type = other RNA
aggtcagtatctaatataa

SEQ ID NO: 127 - RNA, 19 nt, synthetic construct
  source 1..19: mol_type = other RNA
gccaggagctgctagccaa

SEQ ID NO: 128 - RNA, 19 nt, synthetic construct
  source 1..19: mol_type = other RNA
cctttgacgtgtacaagca

SEQ ID NO: 129 - RNA, 19 nt, synthetic construct
  source 1..19: mol_type = other RNA
ctctatgagttgtgacttt

SEQ ID NO: 130 - RNA, 19 nt, synthetic construct
  source 1..19: mol_type = other RNA
gccatatgttgctgggaat

SEQ ID NO: 131 - RNA, 19 nt, synthetic construct
  source 1..19: mol_type = other RNA
ccgcctccattcctactaa

SEQ ID NO: 132 - RNA, 19 nt, synthetic construct
  source 1..19: mol_type = other RNA
gcaaagactatgacagcat

SEQ ID NO: 133 - RNA, 19 nt, synthetic construct
  source 1..19: mol_type = other RNA
agactatgacagcatcaaa

SEQ ID NO: 134 - RNA, 19 nt, synthetic construct
  source 1..19: mol_type = other RNA
gactatgacagcatcaaat

SEQ ID NO: 135 - RNA, 19 nt, synthetic construct
  source 1..19: mol_type = other RNA
actatgacagcatcaaatt

SEQ ID NO: 136 - RNA, 19 nt, synthetic construct
  source 1..19: mol_type = other RNA
ctatgacagcatcaaattt

SEQ ID NO: 137 - RNA, 19 nt, synthetic construct
  source 1..19: mol_type = other RNA
atgacagcatcaaatttca

SEQ ID NO: 138 - RNA, 19 nt, synthetic construct
  source 1..19: mol_type = other RNA
tgacagcatcaaatttcaa

SEQ ID NO: 139 - RNA, 19 nt, synthetic construct
  source 1..19: mol_type = other RNA
cagacagtacaggctagat

SEQ ID NO: 140 - RNA, 19 nt, synthetic construct
  source 1..19: mol_type = other RNA
agacagtacaggctagata

SEQ ID NO: 141 - RNA, 19 nt, synthetic construct
  source 1..19: mol_type = other RNA
gacagtacaggctagataa

SEQ ID NO: 142 - RNA, 19 nt, synthetic construct
  source 1..19: mol_type = other RNA
aaacatttccaataaaaat

SEQ ID NO: 143 - RNA, 19 nt, synthetic construct
  source 1..19: mol_type = other RNA
acatttccaataaaaatat

SEQ ID NO: 144 - RNA, 19 nt, synthetic construct
  source 1..19: mol_type = other RNA
ctctgaaccccagtgactt

SEQ ID NO: 145 - RNA, 19 nt, synthetic construct
  source 1..19: mol_type = other RNA
gacctttccgtgtctgtga

SEQ ID NO: 146 - RNA, 19 nt, synthetic construct
  source 1..19: mol_type = other RNA
cctcacatcccaagtctat

SEQ ID NO: 147 - RNA, 19 nt, synthetic construct
  source 1..19: mol_type = other RNA
ccctaaactccccagcata

SEQ ID NO: 148 - RNA, 19 nt, synthetic construct
  source 1..19: mol_type = other RNA
atttccaataaaaatatca

SEQ ID NO: 149 - RNA, 19 nt, synthetic construct
  source 1..19: mol_type = other RNA
tactcaggtcagtatctaa

SEQ ID NO: 150 - RNA, 19 nt, synthetic construct
  source 1..19: mol_type = other RNA
caccatggagtacctctca

SEQ ID NO: 151 - RNA, 19 nt, synthetic construct
  source 1..19: mol_type = other RNA
aggtcagtatctaatataa

SEQ ID NO: 152 - RNA, 19 nt, synthetic construct
  source 1..19: mol_type = other RNA
ctctatgagttgtgacttt

SEQ ID NO: 153 - RNA, 19 nt, synthetic construct
  source 1..19: mol_type = other RNA
agactatgacagcatcaaa

SEQ ID NO: 154 - RNA, 19 nt, synthetic construct
  source 1..19: mol_type = other RNA
gactatgacagcatcaaat

SEQ ID NO: 155 - RNA, 19 nt, synthetic construct
  source 1..19: mol_type = other RNA
actatgacagcatcaaatt

SEQ ID NO: 156 - RNA, 19 nt, synthetic construct
  source 1..19: mol_type = other RNA
ctatgacagcatcaaattt

SEQ ID NO: 157 - RNA, 19 nt, synthetic construct
  source 1..19: mol_type = other RNA
atgacagcatcaaatttca

SEQ ID NO: 158 - RNA, 19 nt, synthetic construct
  source 1..19: mol_type = other RNA
tgacagcatcaaatttcaa

SEQ ID NO: 159 - RNA, 19 nt, synthetic construct
  source 1..19: mol_type = other RNA
cagacagtacaggctagat

SEQ ID NO: 160 - RNA, 19 nt, synthetic construct
  source 1..19: mol_type = other RNA
agacagtacaggctagata

SEQ ID NO: 161 - RNA, 19 nt, synthetic construct
  source 1..19: mol_type = other RNA
gacagtacaggctagataa

SEQ ID NO: 162 - RNA, 19 nt, synthetic construct
  source 1..19: mol_type = other RNA
aaacatttccaataaaaat

SEQ ID NO: 163 - RNA, 19 nt, synthetic construct
  source 1..19: mol_type = other RNA
acatttccaataaaaatat

SEQ ID NO: 164 - RNA, 19 nt, synthetic construct
  source 1..19: mol_type = other RNA
ccctaaactccccagcata

SEQ ID NO: 165 - RNA, 19 nt, synthetic construct
  source 1..19: mol_type = other RNA
gactatgacagcatcaaaa

SEQ ID NO: 166 - RNA, 19 nt, synthetic construct
  source 1..19: mol_type = other RNA
aaacatttccaataaaaaa

SEQ ID NO: 167 - RNA, 19 nt, synthetic construct
  source 1..19: mol_type = other RNA
acatttccaataaaaataa

SEQ ID NO: 168 - RNA, 19 nt, synthetic construct
  source 1..19: mol_type = other RNA
gctctgaaccccagtgaca

SEQ ID NO: 169 - RNA, 19 nt, synthetic construct
  source 1..19: mol_type = other RNA
gccaggagctgctagccaa

SEQ ID NO: 170 - RNA, 19 nt, synthetic construct
  source 1..19: mol_type = other RNA
cctttgacgtgtacaagca

SEQ ID NO: 171 - RNA, 19 nt, synthetic construct
  source 1..19: mol_type = other RNA
gccatatgttgctgggaaa

SEQ ID NO: 172 - RNA, 19 nt, synthetic construct
  source 1..19: mol_type = other RNA
ccgcctccattcctactaa

SEQ ID NO: 173 - RNA, 19 nt, synthetic construct
  source 1..19: mol_type = other RNA
gcaaagactatgacagcaa

SEQ ID NO: 174 - RNA, 19 nt, synthetic construct
  source 1..19: mol_type = other RNA
ctctgaaccccagtgacta

SEQ ID NO: 175 - RNA, 19 nt, synthetic construct
  source 1..19: mol_type = other RNA
gacctttccgtgtctgtga

SEQ ID NO: 176 - RNA, 19 nt, synthetic construct
  source 1..19: mol_type = other RNA
cctcacatcccaagtctaa

SEQ ID NO: 177 - RNA, 19 nt, synthetic construct
  source 1..19: mol_type = other RNA
atttccaataaaaatatca

SEQ ID NO: 178 - RNA, 21 nt, synthetic construct
  source 1..21: mol_type = other RNA
aaaaacatttccaataaaaaa

SEQ ID NO: 179 - RNA, 21 nt, synthetic construct
  source 1..21: mol_type = other RNA
aaacatttccaataaaaataa

SEQ ID NO: 180 - RNA, 19 nt, synthetic construct
  source 1..19: mol_type = other RNA
acagaacctttcagcataa

SEQ ID NO: 181 - RNA, 19 nt, synthetic construct
  source 1..19: mol_type = other RNA
tgactgctgctacatctaa

SEQ ID NO: 182 - RNA, 19 nt, synthetic construct
  source 1..19: mol_type = other RNA
agcctgactgctgctacat

SEQ ID NO: 183 - RNA, 19 nt, synthetic construct
  source 1..19: mol_type = other RNA
cccttacctgaagaatgct

SEQ ID NO: 184 - RNA, 19 nt, synthetic construct
  source 1..19: mol_type = other RNA
tcacatcccaagtctataa

SEQ ID NO: 185 - RNA, 19 nt, synthetic construct
  source 1..19: mol_type = other RNA
cttacctgaagaatgctgt

SEQ ID NO: 186 - RNA, 19 nt, synthetic construct
  source 1..19: mol_type = other RNA
tatgacagcatcaaattta

SEQ ID NO: 187 - RNA, 19 nt, synthetic construct
  source 1..19: mol_type = other RNA
gcctgactgctgctacata

SEQ ID NO: 188 - RNA, 19 nt, synthetic construct
  source 1..19: mol_type = other RNA
tacccttacctgaagaata

SEQ ID NO: 189 - RNA, 19 nt, synthetic construct
  source 1..19: mol_type = other RNA
ccttacctgaagaatgcta

SEQ ID NO: 190 - RNA, 19 nt, synthetic construct
  source 1..19: mol_type = other RNA
tagataacccacccaattt

SEQ ID NO: 191 - RNA, 19 nt, synthetic construct
  source 1..19: mol_type = other RNA
ctaaactccccagcatact

SEQ ID NO: 192 - RNA, 19 nt, synthetic construct
  source 1..19: mol_type = other RNA
cagcctgactgctgctaca

SEQ ID NO: 193 - RNA, 19 nt, synthetic construct
  source 1..19: mol_type = other RNA
acaaaaacatttccaataa

SEQ ID NO: 194 - RNA, 19 nt, synthetic construct
  source 1..19: mol_type = other RNA
actgctgaatggagtgcta

SEQ ID NO: 195 - RNA, 19 nt, synthetic construct
  source 1..19: mol_type = other RNA
acctttccgtgtctgtgat

SEQ ID NO: 196 - RNA, 19 nt, synthetic construct
  source 1..19: mol_type = other RNA
gacttactcaggtcagtat

SEQ ID NO: 197 - RNA, 19 nt, synthetic construct
  source 1..19: mol_type = other RNA
ctagataacccacccaatt

SEQ ID NO: 198 - RNA, 19 nt, synthetic construct
  source 1..19: mol_type = other RNA
accccagtgacttactcaa

SEQ ID NO: 199 - RNA, 19 nt, synthetic construct
  source 1..19: mol_type = other RNA
gtacctctcagctctgaaa

SEQ ID NO: 200 - RNA, 19 nt, synthetic construct
  source 1..19: mol_type = other RNA
acatcccaagtctatacca

SEQ ID NO: 201 - RNA, 19 nt, synthetic construct
  source 1..19: mol_type = other RNA
agtacaggctagataacca

SEQ ID NO: 202 - RNA, 19 nt, synthetic construct
  source 1..19: mol_type = other RNA
cttactcaggtcagtatct

SEQ ID NO: 203 - RNA, 19 nt, synthetic construct
  source 1..19: mol_type = other RNA
ctcaggtcagtatctaata

SEQ ID NO: 204 - RNA, 19 nt, synthetic construct
  source 1..19: mol_type = other RNA
ccccagaatcattccaaca

SEQ ID NO: 205 - RNA, 19 nt, synthetic construct
  source 1..19: mol_type = other RNA
cagcataacgcctcacata

SEQ ID NO: 206 - RNA, 19 nt, synthetic construct
  source 1..19: mol_type = other RNA
aacaaaaacatttccaata

SEQ ID NO: 207 - RNA, 19 nt, synthetic construct
  source 1..19: mol_type = other RNA
cctaaactccccagcataa

SEQ ID NO: 208 - RNA, 19 nt, synthetic construct
  source 1..19: mol_type = other RNA
aatataagctcggagttta

SEQ ID NO: 209 - RNA, 19 nt, synthetic construct
  source 1..19: mol_type = other RNA
tccctaaactccccagcat

SEQ ID NO: 210 - RNA, 19 nt, synthetic construct
  source 1..19: mol_type = other RNA
cccagtgacttactcaggt

SEQ ID NO: 211 - RNA, 19 nt, synthetic construct
  source 1..19: mol_type = other RNA
gtcagtatctaatataaga

SEQ ID NO: 212 - RNA, 19 nt, synthetic construct
  source 1..19: mol_type = other RNA
tacctctcagctctgaaca

SEQ ID NO: 213 - RNA, 19 nt, synthetic construct
  source 1..19: mol_type = other RNA
taaactccccagcatacta

SEQ ID NO: 214 - RNA, 19 nt, synthetic construct
  source 1..19: mol_type = other RNA
ggtgttgcagtctggtcaa

SEQ ID NO: 215 - RNA, 19 nt, synthetic construct
  source 1..19: mol_type = other RNA
gtgacttactcaggtcagt

SEQ ID NO: 216 - RNA, 19 nt, synthetic construct
  source 1..19: mol_type = other RNA
tgtcaaagccacattctaa

SEQ ID NO: 217 - RNA, 19 nt, synthetic construct
  source 1..19: mol_type = other RNA
ggacttggcccaaagaaaa

SEQ ID NO: 218 - RNA, 19 nt, synthetic construct
  source 1..19: mol_type = other RNA
acagaacctttcagcataa

SEQ ID NO: 219 - RNA, 19 nt, synthetic construct
  source 1..19: mol_type = other RNA
tgactgctgctacatctaa

SEQ ID NO: 220 - RNA, 19 nt, synthetic construct
  source 1..19: mol_type = other RNA
agcctgactgctgctacat

SEQ ID NO: 221 - RNA, 19 nt, synthetic construct
  source 1..19: mol_type = other RNA
cccttacctgaagaatgct

SEQ ID NO: 222 - RNA, 19 nt, synthetic construct
  source 1..19: mol_type = other RNA
tcacatcccaagtctataa

SEQ ID NO: 223 - RNA, 19 nt, synthetic construct
  source 1..19: mol_type = other RNA
cttacctgaagaatgctgt

SEQ ID NO: 224 - RNA, 19 nt, synthetic construct
  source 1..19: mol_type = other RNA
tatgacagcatcaaattta

SEQ ID NO: 225 - RNA, 19 nt, synthetic construct
  source 1..19: mol_type = other RNA
gcctgactgctgctacata

SEQ ID NO: 226 - RNA, 19 nt, synthetic construct
  source 1..19: mol_type = other RNA
tacccttacctgaagaata

SEQ ID NO: 227 - RNA, 19 nt, synthetic construct
  source 1..19: mol_type = other RNA
ccttacctgaagaatgcta

SEQ ID NO: 228 - RNA, 19 nt, synthetic construct
  source 1..19: mol_type = other RNA
tagataacccacccaattt

SEQ ID NO: 229 - RNA, 19 nt, synthetic construct
  source 1..19: mol_type = other RNA
ctaaactccccagcatact

SEQ ID NO: 230 - RNA, 19 nt, synthetic construct
  source 1..19: mol_type = other RNA
cagcctgactgctgctaca

SEQ ID NO: 231 - RNA, 19 nt, synthetic construct
  source 1..19: mol_type = other RNA
acaaaaacatttccaataa

SEQ ID NO: 232 - RNA, 19 nt, synthetic construct
  source 1..19: mol_type = other RNA
actgctgaatggagtgcta

SEQ ID NO: 233 - RNA, 19 nt, synthetic construct
  source 1..19: mol_type = other RNA
acctttccgtgtctgtgat

SEQ ID NO: 234 - RNA, 19 nt, synthetic construct
  source 1..19: mol_type = other RNA
gacttactcaggtcagtat

SEQ ID NO: 235 - RNA, 19 nt, synthetic construct
  source 1..19: mol_type = other RNA
ctagataacccacccaatt

SEQ ID NO: 236 - RNA, 19 nt, synthetic construct
  source 1..19: mol_type = other RNA
accccagtgacttactcaa

SEQ ID NO: 237 - RNA, 19 nt, synthetic construct
  source 1..19: mol_type = other RNA
gtacctctcagctctgaaa

SEQ ID NO: 238 - RNA, 19 nt, synthetic construct
  source 1..19: mol_type = other RNA
acatcccaagtctatacca

SEQ ID NO: 239 - RNA, 19 nt, synthetic construct
  source 1..19: mol_type = other RNA
agtacaggctagataacca

SEQ ID NO: 240 - RNA, 19 nt, synthetic construct
  source 1..19: mol_type = other RNA
cttactcaggtcagtatct

SEQ ID NO: 241 - RNA, 19 nt, synthetic construct
  source 1..19: mol_type = other RNA
ctcaggtcagtatctaata

SEQ ID NO: 242 - RNA, 19 nt, synthetic construct
  source 1..19: mol_type = other RNA
ccccagaatcattccaaca

SEQ ID NO: 243 - RNA, 19 nt, synthetic construct
  source 1..19: mol_type = other RNA
cagcataacgcctcacata

SEQ ID NO: 244 - RNA, 19 nt, synthetic construct
  source 1..19: mol_type = other RNA
aacaaaaacatttccaata

SEQ ID NO: 245 - RNA, 19 nt, synthetic construct
  source 1..19: mol_type = other RNA
cctaaactccccagcataa

SEQ ID NO: 246 - RNA, 19 nt, synthetic construct
  source 1..19: mol_type = other RNA
aatataagctcggagttta

SEQ ID NO: 247 - RNA, 19 nt, synthetic construct
  source 1..19: mol_type = other RNA
tccctaaactccccagcat

SEQ ID NO: 248 - RNA, 19 nt, synthetic construct
  source 1..19: mol_type = other RNA
cccagtgacttactcaggt

SEQ ID NO: 249 - RNA, 19 nt, synthetic construct
  source 1..19: mol_type = other RNA
gtcagtatctaatataaga

SEQ ID NO: 250 - RNA, 19 nt, synthetic construct
  source 1..19: mol_type = other RNA
tacctctcagctctgaaca

SEQ ID NO: 251 - RNA, 19 nt, synthetic construct
  source 1..19: mol_type = other RNA
taaactccccagcatacta

SEQ ID NO: 252 - RNA, 19 nt, synthetic construct
  source 1..19: mol_type = other RNA
ggtgttgcagtctggtcaa

SEQ ID NO: 253 - RNA, 19 nt, synthetic construct
  source 1..19: mol_type = other RNA
gtgacttactcaggtcagt

SEQ ID NO: 254 - RNA, 19 nt, synthetic construct
  source 1..19: mol_type = other RNA
tgtcaaagccacattctaa

SEQ ID NO: 255 - RNA, 19 nt, synthetic construct
  source 1..19: mol_type = other RNA
ggacttggcccaaagaaaa

SEQ ID NO: 256 - RNA, 21 nt, synthetic construct
  source 1..21: mol_type = other RNA
ctatgacagcatcaaatttct

SEQ ID NO: 257 - RNA, 21 nt, synthetic construct
  source 1..21: mol_type = other RNA
tgagaggtactccatggtgga

SEQ ID NO: 258 - RNA, 21 nt, synthetic construct
  source 1..21: mol_type = other RNA
agtcactggggttcagagctg

SEQ ID NO: 259 - RNA, 21 nt, synthetic construct
  source 1..21: mol_type = other RNA
ttagatactgacctgagtaag

SEQ ID NO: 260 - RNA, 21 nt, synthetic construct
  source 1..21: mol_type = other RNA
ttatattagatactgacctga

SEQ ID NO: 261 - RNA, 21 nt, synthetic construct
  source 1..21: mol_type = other RNA
ttggctagcagctcctggctg

SEQ ID NO: 262 - RNA, 21 nt, synthetic construct
  source 1..21: mol_type = other RNA
tgcttgtacacgtcaaaggtg

SEQ ID NO: 263 - RNA, 21 nt, synthetic construct
  source 1..21: mol_type = other RNA
aaagtcacaactcatagagta

SEQ ID NO: 264 - RNA, 21 nt, synthetic construct
  source 1..21: mol_type = other RNA
attcccagcaacatatggctc

SEQ ID NO: 265 - RNA, 21 nt, synthetic construct
  source 1..21: mol_type = other RNA
ttagtaggaatggaggcggtc

SEQ ID NO: 266 - RNA, 21 nt, synthetic construct
  source 1..21: mol_type = other RNA
atgctgtcatagtctttgcag

SEQ ID NO: 267 - RNA, 21 nt, synthetic construct
  source 1..21: mol_type = other RNA
tttgatgctgtcatagtcttt

SEQ ID NO: 268 - RNA, 21 nt, synthetic construct
  source 1..21: mol_type = other RNA
atttgatgctgtcatagtctt

SEQ ID NO: 269 - RNA, 21 nt, synthetic construct
  source 1..21: mol_type = other RNA
aatttgatgctgtcatagtct

SEQ ID NO: 270 - RNA, 21 nt, synthetic construct
  source 1..21: mol_type = other RNA
aaatttgatgctgtcatagtc

SEQ ID NO: 271 - RNA, 21 nt, synthetic construct
  source 1..21: mol_type = other RNA
tgaaatttgatgctgtcatag

SEQ ID NO: 272 - RNA, 21 nt, synthetic construct
  source 1..21: mol_type = other RNA
ttgaaatttgatgctgtcata

SEQ ID NO: 273 - RNA, 21 nt, synthetic construct
  source 1..21: mol_type = other RNA
atctagcctgtactgtctgca

SEQ ID NO: 274 - RNA, 21 nt, synthetic construct
  source 1..21: mol_type = other RNA
tatctagcctgtactgtctgc

SEQ ID NO: 275 - RNA, 21 nt, synthetic construct
  source 1..21: mol_type = other RNA
ttatctagcctgtactgtctg

SEQ ID NO: 276 - RNA, 21 nt, synthetic construct
  source 1..21: mol_type = other RNA
atttttattggaaatgttttt

SEQ ID NO: 277 - RNA, 21 nt, synthetic construct
  source 1..21: mol_type = other RNA
atatttttattggaaatgttt

SEQ ID NO: 278 - RNA, 21 nt, synthetic construct
  source 1..21: mol_type = other RNA
aagtcactggggttcagagct

SEQ ID NO: 279 - RNA, 21 nt, synthetic construct
  source 1..21: mol_type = other RNA
tcacagacacggaaaggtcgc

SEQ ID NO: 280 - RNA, 21 nt, synthetic construct
  source 1..21: mol_type = other RNA
atagacttgggatgtgaggcg

SEQ ID NO: 281 - RNA, 21 nt, synthetic construct
  source 1..21: mol_type = other RNA
tatgctggggagtttagggac

SEQ ID NO: 282 - RNA, 21 nt, synthetic construct
  source 1..21: mol_type = other RNA
tgatatttttattggaaatgt

SEQ ID NO: 283 - RNA, 21 nt, synthetic construct
  source 1..21: mol_type = other RNA
  modified_base 1: mod_base = OTHER; note = t is (SCP-U)
  modified_base 2: mod_base = OTHER; note = t is dT
  modified_base 5: mod_base = OTHER; note = a is dA
  modified_base 7: mod_base = OTHER; note = a is dA
  modified_base 12: mod_base = OTHER; note = c is dC
ttagatactgacctgagtaag

SEQ ID NO: 284 - RNA, 21 nt, synthetic construct
  source 1..21: mol_type = other RNA
  modified_base 1: mod_base = OTHER; note = t is (SCP-U)
  modified_base 2: mod_base = OTHER; note = t is dT
  modified_base 5: mod_base = OTHER; note = a is dA
  modified_base 7: mod_base = OTHER; note = t is dT
  modified_base 12: mod_base = OTHER; note = a is dA
ttatattagatactgacctga

SEQ ID NO: 285 - RNA, 21 nt, synthetic construct
  source 1..21: mol_type = other RNA
  modified_base 1: mod_base = OTHER; note = t is (SCP-U)
  modified_base 2: mod_base = OTHER; note = t is dT
  modified_base 5: mod_base = OTHER; note = a is dA
  modified_base 7: mod_base = OTHER; note = g is dG
  modified_base 12: mod_base = OTHER; note = c is dC
tttgatgctgtcatagtcttt

SEQ ID NO: 286 - RNA, 21 nt, synthetic construct
  source 1..21: mol_type = other RNA
  modified_base 1: mod_base = OTHER; note = t is (SCP-U)
  modified_base 2: mod_base = OTHER; note = t is dT
  modified_base 5: mod_base = OTHER; note = g is dG
  modified_base 7: mod_base = OTHER; note = t is dT
  modified_base 12: mod_base = OTHER; note = t is dT
ttttgatgctgtcatagtctt

SEQ ID NO: 287 - RNA, 21 nt, synthetic construct
  source 1..21: mol_type = other RNA
  modified_base 1: mod_base = OTHER; note = t is (SCP-U)
  modified_base 2: mod_base = OTHER; note = g is dG
  modified_base 5: mod_base = OTHER; note = a is dA
  modified_base 7: mod_base = OTHER; note = t is dT
  modified_base 12: mod_base = OTHER; note = g is dG
tgaaatttgatgctgtcatag

SEQ ID NO: 288 - RNA, 21 nt, synthetic construct
  source 1..21: mol_type = other RNA
  modified_base 1: mod_base = OTHER; note = t is (SCP-U)
  modified_base 2: mod_base = OTHER; note = t is dT
  modified_base 5: mod_base = OTHER; note = a is dA
  modified_base 7: mod_base = OTHER; note = t is dT
  modified_base 12: mod_base = OTHER; note = t is dT
ttgaaatttgatgctgtcata

SEQ ID NO: 289 - RNA, 21 nt, synthetic construct
  source 1..21: mol_type = other RNA
  modified_base 1: mod_base = OTHER; note = t is (SCP-U)
  modified_base 2: mod_base = OTHER; note = a is dA
  modified_base 5: mod_base = OTHER; note = t is dT
  modified_base 7: mod_base = OTHER; note = g is dG
  modified_base 12: mod_base = OTHER; note = t is dT
tatctagcctgtactgtctgc

SEQ ID NO: 290 - RNA, 21 nt, synthetic construct
  source 1..21: mol_type = other RNA
  modified_base 1: mod_base = OTHER; note = t is (SCP-U)
  modified_base 2: mod_base = OTHER; note = t is dT
  modified_base 5: mod_base = OTHER; note = c is dC
  modified_base 7: mod_base = OTHER; note = a is dA
  modified_base 12: mod_base = OTHER; note = g is dG
ttatctagcctgtactgtctg

SEQ ID NO: 291 - RNA, 21 nt, synthetic construct
  source 1..21: mol_type = other RNA
  modified_base 1: mod_base = OTHER; note = t is (SCP-U)
  modified_base 2: mod_base = OTHER; note = t is dT
  modified_base 5: mod_base = OTHER; note = t is dT
  modified_base 7: mod_base = OTHER; note = a is dA
  modified_base 12: mod_base = OTHER; note = a is dA
ttttttattggaaatgttttt

SEQ ID NO: 292 - RNA, 21 nt, synthetic construct
  source 1..21: mol_type = other RNA
  modified_base 1: mod_base = OTHER; note = t is (SCP-U)
  modified_base 2: mod_base = OTHER; note = t is dT
  modified_base 5: mod_base = OTHER; note = t is dT
  modified_base 7: mod_base = OTHER; note = t is dT
  modified_base 12: mod_base = OTHER; note = g is dG
ttatttttattggaaatgttt

SEQ ID NO: 293 - RNA, 21 nt, synthetic construct
  source 1..21: mol_type = other RNA
  modified_base 1: mod_base = OTHER; note = t is (SCP-U)
  modified_base 2: mod_base = OTHER; note = g is dG
  modified_base 5: mod_base = OTHER; note = a is dA
  modified_base 7: mod_base = OTHER; note = t is dT
  modified_base 12: mod_base = OTHER; note = t is dT
tgtcactggggttcagagctg

SEQ ID NO: 294 - RNA, 21 nt, synthetic construct
  source 1..21: mol_type = other RNA
  modified_base 1: mod_base = OTHER; note = t is (SCP-U)
  modified_base 2: mod_base = OTHER; note = t is dT
  modified_base 5: mod_base = OTHER; note = c is dC
  modified_base 7: mod_base = OTHER; note = a is dA
  modified_base 12: mod_base = OTHER; note = c is dC
ttggctagcagctcctggctg

SEQ ID NO: 295 - RNA, 21 nt, synthetic construct
  source 1..21: mol_type = other RNA
  modified_base 1: mod_base = OTHER; note = t is (SCP-U)
  modified_base 2: mod_base = OTHER; note = g is dG
  modified_base 5: mod_base = OTHER; note = t is dT
  modified_base 7: mod_base = OTHER; note = t is dT
  modified_base 12: mod_base = OTHER; note = g is dG
tgcttgtacacgtcaaaggtg

SEQ ID NO: 296 - RNA, 21 nt, synthetic construct
  source 1..21: mol_type = other RNA
  modified_base 1: mod_base = OTHER; note = t is (SCP-U)
  modified_base 2: mod_base = OTHER; note = t is dT
  modified_base 5: mod_base = OTHER; note = c is dC
  modified_base 7: mod_base = OTHER; note = a is dA
  modified_base 12: mod_base = OTHER; note = c is dC
tttcccagcaacatatggctc

SEQ ID NO: 297 - RNA, 21 nt, synthetic construct
  source 1..21: mol_type = other RNA
  modified_base 1: mod_base = OTHER; note = t is (SCP-U)
  modified_base 2: mod_base = OTHER; note = t is dT
  modified_base 5: mod_base = OTHER; note = t is dT
  modified_base 7: mod_base = OTHER; note = g is dG
  modified_base 12: mod_base = OTHER; note = g is dG
ttagtaggaatggaggcggtc

SEQ ID NO: 298 - RNA, 21 nt, synthetic construct
  source 1..21: mol_type = other RNA
  modified_base 1: mod_base = OTHER; note = t is (SCP-U)
  modified_base 2: mod_base = OTHER; note = t is dT
  modified_base 5: mod_base = OTHER; note = t is dT
  modified_base 7: mod_base = OTHER; note = t is dT
  modified_base 12: mod_base = OTHER; note = g is dG
ttgctgtcatagtctttgcag

SEQ ID NO: 299 - RNA, 21 nt, synthetic construct
  source 1..21: mol_type = other RNA
  modified_base 1: mod_base = OTHER; note = t is (SCP-U)
  modified_base 2: mod_base = OTHER; note = a is dA
  modified_base 5: mod_base = OTHER; note = c is dC
  modified_base 7: mod_base = OTHER; note = c is dC
  modified_base 12: mod_base = OTHER; note = g is dG
tagtcactggggttcagagct

SEQ ID NO: 300 - RNA, 21 nt, synthetic construct
  source 1..21: mol_type = other RNA
  modified_base 1: mod_base = OTHER; note = t is (SCP-U)
  modified_base 2: mod_base = OTHER; note = c is dC
  modified_base 5: mod_base = OTHER; note = a is dA
  modified_base 7: mod_base = OTHER; note = a is dA
  modified_base 12: mod_base = OTHER; note = g is dG
tcacagacacggaaaggtcgc

SEQ ID NO: 301 - RNA, 21 nt, synthetic construct
  source 1..21: mol_type = other RNA
  modified_base 1: mod_base = OTHER; note = t is (SCP-U)
  modified_base 2: mod_base = OTHER; note = t is dT
  modified_base 5: mod_base = OTHER; note = a is dA
  modified_base 7: mod_base = OTHER; note = t is dT
  modified_base 12: mod_base = OTHER; note = a is dA
ttagacttgggatgtgaggcg

SEQ ID NO: 302 - RNA, 21 nt, synthetic construct
  source 1..21: mol_type = other RNA
  modified_base 1: mod_base = OTHER; note = t is (SCP-U)
  modified_base 2: mod_base = OTHER; note = g is dG
  modified_base 5: mod_base = OTHER; note = a is dA
  modified_base 7: mod_base = OTHER; note = t is dT
  modified_base 12: mod_base = OTHER; note = t is dT
tgatatttttattggaaatgt

SEQ ID NO: 303 - RNA, 23 nt, synthetic construct
  source 1..23: mol_type = other RNA
  modified_base 1: mod_base = OTHER; note = t is (SCP-U)
ttttttattggaaatgtttttgt

SEQ ID NO: 304 - RNA, 23 nt, synthetic construct
  source 1..23: mol_type = other RNA
  modified_base 1: mod_base = OTHER; note = t is (SCP-U)
ttatttttattggaaatgttttt

SEQ ID NO: 305 - RNA, 21 nt, synthetic construct
  source 1..21: mol_type = other RNA
ttatgctgaaaggttctgtca

SEQ ID NO: 306 - RNA, 21 nt, synthetic construct
  source 1..21: mol_type = other RNA
ttagatgtagcagcagtcagg

SEQ ID NO: 307 - RNA, 21 nt, synthetic construct
  source 1..21: mol_type = other RNA
atgtagcagcagtcaggctgg

SEQ ID NO: 308 - RNA, 21 nt, synthetic construct
  source 1..21: mol_type = other RNA
agcattcttcaggtaagggta

SEQ ID NO: 309 - RNA, 21 nt, synthetic construct
  source 1..21: mol_type = other RNA
ttatagacttgggatgtgagg

SEQ ID NO: 310 - RNA, 21 nt, synthetic construct
  source 1..21: mol_type = other RNA
acagcattcttcaggtaaggg

SEQ ID NO: 311 - RNA, 21 nt, synthetic construct
  source 1..21: mol_type = other RNA
taaatttgatgctgtcatagt

SEQ ID NO: 312 - RNA, 21 nt, synthetic construct
  source 1..21: mol_type = other RNA
tatgtagcagcagtcaggctg

SEQ ID NO: 313 - RNA, 21 nt, synthetic construct
  source 1..21: mol_type = other RNA
tattcttcaggtaagggtata

SEQ ID NO: 314 - RNA, 21 nt, synthetic construct
  source 1..21: mol_type = other RNA
tagcattcttcaggtaagggt

SEQ ID NO: 315 - RNA, 21 nt, synthetic construct
  source 1..21: mol_type = other RNA
aaattgggtgggttatctagc

SEQ ID NO: 316 - RNA, 21 nt, synthetic construct
  source 1..21: mol_type = other RNA
agtatgctggggagtttaggg

SEQ ID NO: 317 - RNA, 21 nt, synthetic construct
  source 1..21: mol_type = other RNA
tgtagcagcagtcaggctggg

SEQ ID NO: 318 - RNA, 21 nt, synthetic construct
  source 1..21: mol_type = other RNA
ttattggaaatgtttttgtta

SEQ ID NO: 319 - RNA, 21 nt, synthetic construct
  source 1..21: mol_type = other RNA
tagcactccattcagcagtag

SEQ ID NO: 320 - RNA, 21 nt, synthetic construct
  source 1..21: mol_type = other RNA
atcacagacacggaaaggtcg

SEQ ID NO: 321 - RNA, 21 nt, synthetic construct
  source 1..21: mol_type = other RNA
atactgacctgagtaagtcac

SEQ ID NO: 322 - RNA, 21 nt, synthetic construct
  source 1..21: mol_type = other RNA
aattgggtgggttatctagcc

SEQ ID NO: 323 - RNA, 21 nt, synthetic construct
  source 1..21: mol_type = other RNA
ttgagtaagtcactggggttc

SEQ ID NO: 324 - RNA, 21 nt, synthetic construct
  source 1..21: mol_type = other RNA
tttcagagctgagaggtactc

SEQ ID NO: 325 - RNA, 21 nt, synthetic construct
  source 1..21: mol_type = other RNA
tggtatagacttgggatgtga

SEQ ID NO: 326 - RNA, 21 nt, synthetic construct
  source 1..21: mol_type = other RNA
tggttatctagcctgtactgt

SEQ ID NO: 327 - RNA, 21 nt, synthetic construct
  source 1..21: mol_type = other RNA
agatactgacctgagtaagtc

SEQ ID NO: 328 - RNA, 21 nt, synthetic construct
  source 1..21: mol_type = other RNA
tattagatactgacctgagta

SEQ ID NO: 329 - RNA, 21 nt, synthetic construct
  source 1..21: mol_type = other RNA
tgttggaatgattctgggggc

SEQ ID NO: 330 - RNA, 21 nt, synthetic construct
  source 1..21: mol_type = other RNA
tatgtgaggcgttatgctgaa

SEQ ID NO: 331 - RNA, 21 nt, synthetic construct
  source 1..21: mol_type = other RNA
tattggaaatgtttttgttag

SEQ ID NO: 332 - RNA, 21 nt, synthetic construct
  source 1..21: mol_type = other RNA
ttatgctggggagtttaggga

SEQ ID NO: 333 - RNA, 21 nt, synthetic construct
  source 1..21: mol_type = other RNA
taaactccgagcttatattag

SEQ ID NO: 334 - RNA, 21 nt, synthetic construct
  source 1..21: mol_type = other RNA
atgctggggagtttagggaca

SEQ ID NO: 335 - RNA, 21 nt, synthetic construct
  source 1..21: mol_type = other RNA
acctgagtaagtcactggggt

SEQ ID NO: 336 - RNA, 21 nt, synthetic construct
  source 1..21: mol_type = other RNA
tcttatattagatactgacct

SEQ ID NO: 337 - RNA, 21 nt, synthetic construct
  source 1..21: mol_type = other RNA
tgttcagagctgagaggtact

SEQ ID NO: 338 - RNA, 21 nt, synthetic construct
  source 1..21: mol_type = other RNA
tagtatgctggggagtttagg

SEQ ID NO: 339 - RNA, 21 nt, synthetic construct
  source 1..21: mol_type = other RNA
ttgaccagactgcaacaccat

SEQ ID NO: 340 - RNA, 21 nt, synthetic construct
  source 1..21: mol_type = other RNA
actgacctgagtaagtcactg

SEQ ID NO: 341 - RNA, 21 nt, synthetic construct
  source 1..21: mol_type = other RNA
ttagaatgtggctttgacatt

SEQ ID NO: 342 - RNA, 21 nt, synthetic construct
  source 1..21: mol_type = other RNA
ttttctttgggccaagtcctt

SEQ ID NO: 343 - RNA, 21 nt, synthetic construct
  source 1..21: mol_type = other RNA
ttatgctgaaaggttctgtca

SEQ ID NO: 344 - RNA, 21 nt, synthetic construct
  source 1..21: mol_type = other RNA
ttagatgtagcagcagtcagg

SEQ ID NO: 345 - RNA, 21 nt, synthetic construct
  source 1..21: mol_type = other RNA
atgtagcagcagtcaggctgg

SEQ ID NO: 346 - RNA, 21 nt, synthetic construct
  source 1..21: mol_type = other RNA
agcattcttcaggtaagggta

SEQ ID NO: 347 - RNA, 21 nt, synthetic construct
  source 1..21: mol_type = other RNA
ttatagacttgggatgtgagg

SEQ ID NO: 348 - RNA, 21 nt, synthetic construct
  source 1..21: mol_type = other RNA
acagcattcttcaggtaaggg

SEQ ID NO: 349 - RNA, 21 nt, synthetic construct
  source 1..21: mol_type = other RNA
taaatttgatgctgtcatagt

SEQ ID NO: 350 - RNA, 21 nt, synthetic construct
  source 1..21: mol_type = other RNA
tatgtagcagcagtcaggctg

SEQ ID NO: 351 - RNA, 21 nt, synthetic construct
  source 1..21: mol_type = other RNA
tattcttcaggtaagggtata

SEQ ID NO: 352 - RNA, 21 nt, synthetic construct
  source 1..21: mol_type = other RNA
tagcattcttcaggtaagggt

SEQ ID NO: 353 - RNA, 21 nt, synthetic construct
  source 1..21: mol_type = other RNA
aaattgggtgggttatctagc

SEQ ID NO: 354 - RNA, 21 nt, synthetic construct
  source 1..21: mol_type = other RNA
agtatgctggggagtttaggg

SEQ ID NO: 355 - RNA, 21 nt, synthetic construct
  source 1..21: mol_type = other RNA
tgtagcagcagtcaggctggg

SEQ ID NO: 356 - RNA, 21 nt, synthetic construct
  source 1..21: mol_type = other RNA
ttattggaaatgtttttgtta

SEQ ID NO: 357 - RNA, 21 nt, synthetic construct
  source 1..21: mol_type = other RNA
tagcactccattcagcagtag

SEQ ID NO: 358 - RNA, 21 nt, synthetic construct
  source 1..21: mol_type = other RNA
atcacagacacggaaaggtcg

SEQ ID NO: 359 - RNA, 21 nt, synthetic construct
  source 1..21: mol_type = other RNA
atactgacctgagtaagtcac

SEQ ID NO: 360 - RNA, 21 nt, synthetic construct
  source 1..21: mol_type = other RNA
aattgggtgggttatctagcc

SEQ ID NO: 361 - RNA, 21 nt, synthetic construct
  source 1..21: mol_type = other RNA
ttgagtaagtcactggggttc

SEQ ID NO: 362 - RNA, 21 nt, synthetic construct
  source 1..21: mol_type = other RNA
tttcagagctgagaggtactc

SEQ ID NO: 363 - RNA, 21 nt, synthetic construct
  source 1..21: mol_type = other RNA
tggtatagacttgggatgtga

SEQ ID NO: 364 - RNA, 21 nt, synthetic construct
  source 1..21: mol_type = other RNA
tggttatctagcctgtactgt

SEQ ID NO: 365 - RNA, 21 nt, synthetic construct
  source 1..21: mol_type = other RNA
agatactgacctgagtaagtc

SEQ ID NO: 366 - RNA, 21 nt, synthetic construct
  source 1..21: mol_type = other RNA
tattagatactgacctgagta

SEQ ID NO: 367 - RNA, 21 nt, synthetic construct
  source 1..21: mol_type = other RNA
tgttggaatgattctgggggc

SEQ ID NO: 368 - RNA, 21 nt, synthetic construct
  source 1..21: mol_type = other RNA
tatgtgaggcgttatgctgaa

SEQ ID NO: 369 - RNA, 21 nt, synthetic construct
  source 1..21: mol_type = other RNA
tattggaaatgtttttgttag

SEQ ID NO: 370 - RNA, 21 nt, synthetic construct
  source 1..21: mol_type = other RNA
ttatgctggggagtttaggga

SEQ ID NO: 371 - RNA, 21 nt, synthetic construct
  source 1..21: mol_type = other RNA
taaactccgagcttatattag

SEQ ID NO: 372 - RNA, 21 nt, synthetic construct
  source 1..21: mol_type = other RNA
atgctggggagtttagggaca

SEQ ID NO: 373 - RNA, 21 nt, synthetic construct
  source 1..21: mol_type = other RNA
acctgagtaagtcactggggt

SEQ ID NO: 374 - RNA, 21 nt, synthetic construct
  source 1..21: mol_type = other RNA
tcttatattagatactgacct

SEQ ID NO: 375 - RNA, 21 nt, synthetic construct
  source 1..21: mol_type = other RNA
tgttcagagctgagaggtact

SEQ ID NO: 376 - RNA, 21 nt, synthetic construct
  source 1..21: mol_type = other RNA
tagtatgctggggagtttagg

SEQ ID NO: 377 - RNA, 21 nt, synthetic construct
  source 1..21: mol_type = other RNA
ttgaccagactgcaacaccat

SEQ ID NO: 378 - RNA, 21 nt, synthetic construct
  source 1..21: mol_type = other RNA
actgacctgagtaagtcactg

SEQ ID NO: 379 - RNA, 21 nt, synthetic construct
  source 1..21: mol_type = other RNA
ttagaatgtggctttgacatt

SEQ ID NO: 380 - RNA, 21 nt, synthetic construct
  source 1..21: mol_type = other RNA
ttttctttgggccaagtcctt

SEQ ID NO: 381 - RNA, 23 nt, synthetic construct
  source 1..23: mol_type = other RNA
  modified_base 2: mod_base = OTHER; note = g is dG
  modified_base 5: mod_base = OTHER; note = a is dA
  modified_base 7: mod_base = OTHER; note = t is dT
  modified_base 12: mod_base = OTHER; note = g is dG
agaaatttgatgctgtcatagtc

SEQ ID NO: 382 - DNA, 20 bp, synthetic construct
  source 1..20: mol_type = other DNA
acgtggacatccgcaaagac

SEQ ID NO: 383 - DNA, 20 bp, synthetic construct
  source 1..20: mol_type = other DNA
tcttcattgtgctgggtgcc

SEQ ID NO: 384 - DNA, 25 bp, synthetic construct
  source 1..25: mol_type = other DNA
aacacagtgctgtctggcggcacca

SEQ ID NO: 385 - DNA, 20 bp, synthetic construct
  source 1..20: mol_type = other DNA
agccctacaaggagtggagt

SEQ ID NO: 386 - DNA, 20 bp, synthetic construct
  source 1..20: mol_type = other DNA
gagcccgtagaatgtggctt

SEQ ID NO: 387 - DNA, 28 bp, synthetic construct
  source 1..28: mol_type = other DNA
atggcctgggacgggagaggcccaagca

SEQ ID NO: 388 - DNA, 19 bp, synthetic construct
  source 1..19: mol_type = other DNA
ccttccttcctgggcatgg